European Patent Application EP 4 219 749 A2, published August 2, 2023. Title: SPLIT-CYCLE AND TAPE AMPLIFICATION. Applicant: Bio-Rad Laboratories, Inc. Application EP. The sequence listing filed with the application follows.

SEQUENCE LISTING (36 sequences)

SEQ ID NO: 1 - DNA, 68 bp, synthetic construct
  misc_feature 1..68: note = synthetic construct
  source 1..68: mol_type = other DNA
aggcactcttgcctacgccaccagctccaactaccacaagtttatattcagtcattttcagcaggcct

SEQ ID NO: 2 - DNA, 40 bp, synthetic construct
  misc_feature 1..40: note = synthetic construct
  source 1..40: mol_type = other DNA
ctaggagtggctggaatcatggcacgagatcctctctctg

SEQ ID NO: 3 - DNA, 44 bp, synthetic construct
  misc_feature 1..44: note = synthetic construct
  source 1..44: mol_type = other DNA
cctgataacactgatctagcctcgtactcctgctcagtgatttc

SEQ ID NO: 4 - DNA, 44 bp, synthetic construct
  misc_feature 1..44: note = synthetic construct
  source 1..44: mol_type = other DNA
caagcagaagacggcatacgagatgtcacgagatcctctctcta

SEQ ID NO: 5 - DNA, 45 bp, synthetic construct
  misc_feature 1..45: note = synthetic construct
  source 1..45: mol_type = other DNA
ttactatgccgctggtggctctagatgctcctgctcagtgatttt

SEQ ID NO: 6 - DNA, 22 bp, synthetic construct
  misc_feature 1..22: note = synthetic construct
  source 1..22: mol_type = other DNA
ctaggagtggctggaatcatgg

SEQ ID NO: 7 - DNA, 18 bp, synthetic construct
  misc_feature 1..18: note = synthetic construct
  source 1..18: mol_type = other DNA
gattccagacactcctag

SEQ ID NO: 8 - DNA, 26 bp, synthetic construct
  misc_feature 1..26: note = synthetic construct
  source 1..26: mol_type = other DNA
cctgataacactgatctagcctcgta

SEQ ID NO: 9 - DNA, 26 bp, synthetic construct
  misc_feature 1..26: note = synthetic construct
  source 1..26: mol_type = other DNA
caagcagaagacggcatacgagatgt

SEQ ID NO: 10 - DNA, 18 bp, synthetic construct
  misc_feature 1..18: note = synthetic construct
  source 1..18: mol_type = other DNA
gtatgccgtattctgctt

SEQ ID NO: 11 - DNA, 27 bp, synthetic construct
  misc_feature 1..27: note = synthetic construct
  source 1..27: mol_type = other DNA
ttactatgccgctggtggctctagatg

SEQ ID NO: 12 - DNA, 60 bp, synthetic construct
  misc_feature 1..60: note = synthetic construct
  misc_feature 1..10: note = n = any nucleotide
  misc_feature 46..60: note = n = any nucleotide
  source 1..60: mol_type = other DNA
nnnnnnnnnngaggacgagtcactaaacagagagaggatctcgtgnnnnnnnnnnnnnnn

SEQ ID NO: 13 - DNA, 66 bp, synthetic construct
  misc_feature 1..66: note = synthetic construct
  misc_feature 1..13: note = n = any nucleotide
  misc_feature 48..66: note = n = any nucleotide
  source 1..66: mol_type = other DNA
nnnnnnnnnnnnngaggacgagtcactaaatagagagaggatctcgtnnnnnnnnnnnnnnnnnnn

SEQ ID NO: 14 - DNA, 26 bp, synthetic construct
  misc_feature 1..26: note = synthetic construct
  source 1..26: mol_type = other DNA
gaatcatggcttgtggtagttggagc

SEQ ID NO: 15 - DNA, 28 bp, synthetic construct
  misc_feature 1..28: note = synthetic construct
  source 1..28: mol_type = other DNA
ctagcctcgtacttgcctacgccaccag

SEQ ID NO: 16 - DNA, 29 bp, synthetic construct
  misc_feature 1..29: note = synthetic construct
  source 1..29: mol_type = other DNA
catacgagatgtcttgtggtagttggagg

SEQ ID NO: 17 - DNA, 23 bp, synthetic construct
  misc_feature 1..23: note = synthetic construct
  source 1..23: mol_type = other DNA
ctctagatggcctacgccaccac

SEQ ID NO: 18 - skipped

SEQ ID NO: 19 - DNA, 11 bp, synthetic construct
  misc_feature 1..11: note = synthetic construct
  source 1..11: mol_type = other DNA
ctagcctcgta

SEQ ID NO: 20 - DNA, 12 bp, synthetic construct
  misc_feature 1..12: note = synthetic construct
  source 1..12: mol_type = other DNA
catacgagatgt

SEQ ID NO: 21 - DNA, 10 bp, synthetic construct
  misc_feature 1..10: note = synthetic construct
  source 1..10: mol_type = other DNA
gctctagatg

SEQ ID NO: 22 - DNA, 15 bp, synthetic construct
  misc_feature 1..15: note = synthetic construct
  source 1..15: mol_type = other DNA
ttggagctggtggcg

SEQ ID NO: 23 - DNA, 16 bp, synthetic construct
  misc_feature 1..16: note = synthetic construct
  source 1..16: mol_type = other DNA
gtagttggaggtggtg

SEQ ID NO: 24 - DNA, 68 bp, synthetic construct
  misc_feature 1..68: note = synthetic construct
  source 1..68: mol_type = other DNA
aggcactcttgcctacgccaccacctccaactaccacaagtttatattcagtcattttcagcaggcct

SEQ ID NO: 25 - DNA, 37 bp, synthetic construct
  misc_feature 1..37: note = synthetic construct
  source 1..37: mol_type = other DNA
cctgataacactgatctagcctcgtacttgcctacgc

SEQ ID NO: 26 - DNA, 37 bp, synthetic construct
  misc_feature 1..37: note = synthetic construct
  source 1..37: mol_type = other DNA
gtacgaggctagatcatgttatcaggcttgtggtagt

SEQ ID NO: 27 - DNA, 17 bp, synthetic construct
  misc_feature 1..17: note = synthetic construct
  source 1..17: mol_type = other DNA
caccagctccaactacc

SEQ ID NO: 28 - DNA, 68 bp, synthetic construct
  misc_feature 1..68: note = synthetic construct
  source 1..68: mol_type = other DNA
aggcctgctgaaaatgactgaatataaacttgtggtagttggagctggtggcgtaggcaagagtgcct

SEQ ID NO: 29 - DNA, 38 bp, synthetic construct
  misc_feature 1..38: note = synthetic construct
  source 1..38: mol_type = other DNA
gtacgaggctagatcagtgttatcaggcttgtggtagt

SEQ ID NO: 30 - DNA, 87 bp, synthetic construct
  misc_feature 1..87: note = synthetic construct
  source 1..87: mol_type = other DNA
cctgataacactgatctagcctcgtacttgcctacgccaccagctccaactaccacaagtttatattcagtcattttcagcaggcct

SEQ ID NO: 31 - DNA, 86 bp, synthetic construct
  misc_feature 1..86: note = synthetic construct
  source 1..86: mol_type = other DNA
gtacgaggctagatcagtgttatcaggcttgtggtagttggagctggtggcgtaggcaagtacgaggctagatcagtgttatcagg

SEQ ID NO: 32 - DNA, 86 bp, synthetic construct
  misc_feature 1..86: note = synthetic construct
  source 1..86: mol_type = other DNA
cctgataacactgatctagcctcgtacttgcctacgccaccagctccaactaccacaagcctgataacactgatctagcctcgtac

SEQ ID NO: 33 - DNA, 43 bp, synthetic construct
  misc_feature 1..43: note = synthetic construct
  source 1..43: mol_type = other DNA
cctgataacactgatctagcctcgtacttgcctacgccaccag

SEQ ID NO: 34 - DNA, 44 bp, synthetic construct
  misc_feature 1..44: note = synthetic construct
  source 1..44: mol_type = other DNA
gtacgaggctagatcagtgttatcaggcttgtggtagttggagc

SEQ ID NO: 35 - DNA, 10 bp, synthetic construct
  misc_feature 1..10: note = synthetic construct
  source 1..10: mol_type = other DNA
ggactattgt

SEQ ID NO: 36 - DNA, 43 bp, synthetic construct
  misc_feature 1..43: note = synthetic construct
  source 1..43: mol_type = other DNA
gtacgaggctagatcatgttatcaggcttgtggtagttggagc